European Patent Specification EP 3 763 725 B1, published March 5, 2025. Title: BIOMIMETIC PEPTIDES DERIVED FROM BIOLOGICAL SOURCE AND THEIR USES IN RETARDING AGING AND IMPROVING SKIN. Applicant: TCI CO., LTD. The sequence listing filed with the application follows.

SEQUENCE LISTING (15 sequences)

SEQ ID NO: 1 - protein, 4 aa, Artificial Sequence
  Artificial peptide
  MISC_FEATURE (1)..(1): Wherein the amino acid is selected from an amino acid having a positively charged side chain
  MISC_FEATURE (2)..(2): Wherein the amino acid is selected from an amino acid having an uncharged side chain
  MISC_FEATURE (3)..(3): Wherein the amino acid is selected from an amino acid having an uncharged side chain
  MISC_FEATURE (4)..(4): Wherein the amino acid is selected from an amino acid having a positively charged side chain
XXXX

SEQ ID NO: 2 - protein, 4 aa, Artificial Sequence
  Artificial peptide
RTCK

SEQ ID NO: 3 - protein, 4 aa, Artificial Sequence
  Artificial peptide
KSGR

SEQ ID NO: 4 - protein, 4 aa, Artificial Sequence
  Artificial peptide
KSGK

SEQ ID NO: 5 - protein, 4 aa, Artificial Sequence
  Artificial peptide
KYIK

SEQ ID NO: 6 - protein, 4 aa, Artificial Sequence
  Artificial peptide
KIFK

SEQ ID NO: 7 - protein, 4 aa, Artificial Sequence
  Artificial peptide
RPIK

SEQ ID NO: 8 - protein, 4 aa, Artificial Sequence
  Artificial peptide
KNAK

SEQ ID NO: 9 - protein, 5 aa, Artificial Sequence
  Artificial peptide
LKSGR

SEQ ID NO: 10 - protein, 5 aa, Artificial Sequence
  Artificial peptide
KIFKF

SEQ ID NO: 11 - protein, 5 aa, Artificial Sequence
  Artificial peptide
PRPIK

SEQ ID NO: 12 - protein, 6 aa, Artificial Sequence
  Artificial peptide
TKSGKF

SEQ ID NO: 13 - protein, 6 aa, Artificial Sequence
  Artificial peptide
VKNAKY

SEQ ID NO: 14 - protein, 7 aa, Artificial Sequence
  Artificial peptide
QKRRTCK

SEQ ID NO: 15 - protein, 8 aa, Artificial Sequence
  Artificial peptide
QRIKYIKP